European Patent Application EP 4 640 712 A1, published October 29, 2025. Title: Anti-PD-L1 antibody and use thereof. Applicant: HEFEI TG IMMUNOPHARMA CO., LTD. The sequence listing filed with the application follows.

SEQUENCE LISTING (32 sequences)

SEQ ID NO: 1 - protein, 8 aa, synthetic construct
GYSFTGYY

SEQ ID NO: 2 - protein, 8 aa, synthetic construct
INPYNGAT

SEQ ID NO: 3 - protein, 12 aa, synthetic construct
VPTGMGYFLMDY

SEQ ID NO: 4 - protein, 6 aa, synthetic construct
QDVGSA

SEQ ID NO: 5 - protein, 8 aa, synthetic construct
QQFTSYPT

SEQ ID NO: 6 - protein, 119 aa, synthetic construct
EVQLQQSGPDLVKPGASVKISCKASGYSFTGYYMHWVKQSHVKSLEWIGRINPYNGATTYSQNFKDKASLTVDKSSSTAYMELHSLTSEDSAVYYCVPTGMGYFLMDYWGQGTSVTVSS

SEQ ID NO: 7 - protein, 106 aa, synthetic construct
DIVMTQSHKFMSASVGDRVSITCKASQDVGSAVVWYRQKPGQSPKLLIYWASTRHTGVPDRFTGSGSGTDFTLTISNVQSEDLADYFCQQFTSYPTFGSGTRLEIK

SEQ ID NO: 8 - protein, 119 aa, synthetic construct
QVQLVQSGAEVKKPGASVKVSCKASGYSFTGYYMHWVRQAPGQGLEWIGRINPYNGATTYSQNFKDRATMTVDTSISTAYMELSRLRSDDTAVYYCVPTGMGYFLMDYWGQGTLVTVSS

SEQ ID NO: 9 - protein, 106 aa, synthetic construct
DIQLTQSPSFLSASVGDRVTITCKASQDVGSAVVWYQQKPGKAPKLLIYWASTRHTGVPSRFSGSGSGTEFTLTISSLQPEDFATYFCQQFTSYPTFGQGTKLEIK

SEQ ID NO: 10 - protein, 443 aa, synthetic construct
EVQLQQSGPDLVKPGASVKISCKASGYSFTGYYMHWVKQSHVKSLEWIGRINPYNGATTYSQNFKDKASLTVDKSSSTAYMELHSLTSEDSAVYYCVPTGMGYFLMDYWGQGTSVTVSSAKTTPPSVYPLAPGSAAQTNSMVTLGCLVKGYFPEPVTVTWNSGSLSSGVHTFPAVLQSDLYTLSSSVTVPSSPRPSETVTCNVAHPASSTKVDKKIVPRDCGCKPCICTVPEVSSVFIFPPKPKDVLTITLTPKVTCVVVDISKDDPEVQFSWFVDDVEVHTAQTQPREEQFNSTFRSVSELPIMHQDWLNGKEFKCRVNSAAFPAPIEKTISKTKGRPKAPQVYTIPPPKEQMAKDKVSLTCMITDFFPEDITVEWQWNGQPAENYKNTQPIMNTNGSYFVYSKLNVQKSNWEAGNTFTCSVLHEGLHNHHTEKSLSHSPGK

SEQ ID NO: 11 - protein, 213 aa, synthetic construct
DIVMTQSHKFMSASVGDRVSITCKASQDVGSAVVWYRQKPGQSPKLLIYWASTRHTGVPDRFTGSGSGTDFTLTISNVQSEDLADYFCQQFTSYPTFGSGTRLEIKRADAAPTVSIFPPSSEQLTSGGASVVCFLNNFYPKDINVKWKIDGSERQNGVLNSWTDQDSKDSTYSMSSTLTLTKDEYERHNSYTCEATHKTSTSPIVKSFNRNEC

SEQ ID NO: 12 - protein, 449 aa, synthetic construct
QVQLVQSGAEVKKPGASVKVSCKASGYSFTGYYMHWVRQAPGQGLEWIGRINPYNGATTYSQNFKDRATMTVDTSISTAYMELSRLRSDDTAVYYCVPTGMGYFLMDYWGQGTLVTVSSASTKGPSVFPLAPSSKSTSGGTAALGCLVKDYFPEPVTVSWNSGALTSGVHTFPAVLQSSGLYSLSSVVTVPSSSLGTQTYICNVNHKPSNTKVDKKVEPKSCDKTHTCPPCPAPEAAGGPSVFLFPPKPKDTLMISRTPEVTCVVVDVSHEDPEVKFNWYVDGVEVHNAKTKPREEQYNSTYRVVSVLTVLHQDWLNGKEYKCKVSNKALPAPIEKTISKAKGQPREPQVYTLPPSREEMTKNQVSLTCLVKGFYPSDIAVEWESNGQPENNYKTTPPVLDSDGSFFLYSKLTVDKSRWQQGNVFSCSVMHEALHNHYTQKSLSLSPGK

SEQ ID NO: 13 - protein, 213 aa, synthetic construct
DIQLTQSPSFLSASVGDRVTITCKASQDVGSAVVWYQQKPGKAPKLLIYWASTRHTGVPSRFSGSGSGTEFTLTISSLQPEDFATYFCQQFTSYPTFGQGTKLEIKRTVAAPSVFIFPPSDEQLKSGTASVVCLLNNFYPREAKVQWKVDNALQSGNSQESVTEQDSKDSTYSLSSTLTLSKADYEKHKVYACEVTHQGLSSPVTKSFNRGEC

SEQ ID NO: 14 - protein, 288 aa, synthetic construct
MQIPQAPWPVVWAVLQLGWRPGWFLDSPDRPWNPPTFSPALLVVTEGDNATFTCSFSNTSESFVLNWYRMSPSNQTDKLAAFPEDRSQPGQDCRFRVTQLPNGRDFHMSVVRARRNDSGTYLCGAISLAPKAQIKESLRAELRVTERRAEVPTAHPSPSPRPAGQFQTLVVGVVGGLLGSLVLLVWVLAVICSRAARGTIGARRTGQPLKEDPSAVPVFSVDYGELDFQWREKTPEPPVPCVPEQTEYATIVFPSGMGTSSPARRGSADGPRSAQPLRPEDGHCSWPL

SEQ ID NO: 15 - protein, 8 aa, synthetic construct
GFTFNTYA

SEQ ID NO: 16 - protein, 10 aa, synthetic construct
IRSKYNNYAT

SEQ ID NO: 17 - protein, 16 aa, synthetic construct
VRHGNFGNSYVSWFAY

SEQ ID NO: 18 - protein, 9 aa, synthetic construct
TGAVTTSNY

SEQ ID NO: 19 - protein, 9 aa, synthetic construct
ALWYSNLWV

SEQ ID NO: 20 - protein, 125 aa, synthetic construct
EVQLLESGGGLVQPGGSLKLSCAASGFTFNTYAMNWVRQAPGKGLEWVARIRSKYNNYATYYADSVKDRFTISRDDSKNTAYLQMNNLKTEDTAVYYCVRHGNFGNSYVSWFAYWGQGTLVTVSS

SEQ ID NO: 21 - protein, 109 aa, synthetic construct
ELVVTQEPSLTVSPGGTVTLTCRSSTGAVTTSNYANWVQQKPGQAPRGLIGGTNKRAPGTPARFSGSLLGGKAALTLSGVQPEDEAEYYCALWYSNLWVFGGGTKLTVL

SEQ ID NO: 22 - protein, 249 aa, synthetic construct
EVQLLESGGGLVQPGGSLKLSCAASGFTFNTYAMNWVRQAPGKGLEWVARIRSKYNNYATYYADSVKDRFTISRDDSKNTAYLQMNNLKTEDTAVYYCVRHGNFGNSYVSWFAYWGQGTLVTVSSGGGGSGGGGSGGGGSELVVTQEPSLTVSPGGTVTLTCRSSTGAVTTSNYANWVQQKPGQAPRGLIGGTNKRAPGTPARFSGSLLGGKAALTLSGVQPEDEAEYYCALWYSNLWVFGGGTKLTVL

SEQ ID NO: 23 - protein, 449 aa, synthetic construct
QVQLVQSGAEVKKPGASVKVSCKASGYSFTGYYMHWVRQAPGQGLEWIGRINPYNGATTYSQNFKDRATMTVDTSISTAYMELSRLRSDDTAVYYCVPTGMGYFLMDYWGQGTLVTVSSASTKGPSVFPLAPSSKSTSGGTAALGCLVKDYFPEPVTVSWNSGALTSGVHTFPAVLQSSGLYSLSSVVTVPSSSLGTQTYICNVNHKPSNTKVDKKVEPKSCDKTHTCPPCPAPEAAGGPSVFLFPPKPKDTLMISRTPEVTCVVVDVSHEDPEVKFNWYVDGVEVHNAKTKPREEQYNSTYRVVSVLTVLHQDWLNGKEYKCKVSNKALPAPIEKTISKAKGQPREPQVCTLPPSREEMTKNQVSLSCAVKGFYPSDIAVEWESNGQPENNYKTTPPVLDSDGSFFLVSKLTVDKSRWQQGNVFSCSVMHEALHNHYTQKSLSLSPGK

SEQ ID NO: 24 - protein, 485 aa, synthetic construct
EVQLLESGGGLVQPGGSLKLSCAASGFTFNTYAMNWVRQAPGKGLEWVARIRSKYNNYATYYADSVKDRFTISRDDSKNTAYLQMNNLKTEDTAVYYCVRHGNFGNSYVSWFAYWGQGTLVTVSSGGGGSGGGGSGGGGSELVVTQEPSLTVSPGGTVTLTCRSSTGAVTTSNYANWVQQKPGQAPRGLIGGTNKRAPGTPARFSGSLLGGKAALTLSGVQPEDEAEYYCALWYSNLWVFGGGTKLTVLGGGGSPKSSDKTHTCPPCPAPEAAGGPSVFLFPPKPKDTLMISRTPEVTCVVVDVSHEDPEVKFNWYVDGVEVHNAKTKPREEQYNSTYRVVSVLTVLHQDWLNGKEYKCKVSNKALPAPIEKTISKAKGQPREPQVYTLPPCREEMTKNQVSLWCLVKGFYPSDIAVEWESNGQPENNYKTTPPVLDSDGSFFLYSKLTVDKSRWQQGNVFSCSVMHEALHNHYTQKSLSLSPGK

SEQ ID NO: 25 - protein, 449 aa, synthetic construct
QVQLVQSGAEVKKPGASVKVSCKASGYSFTGYYMHWVRQAPGQGLEWIGRINPYNGATTYSQNFKDRATMTVDTSISTAYMELSRLRSDDTAVYYCVPTGMGYFLMDYWGQGTLVTVSSASTKGPSVFPLAPSSKSTSGGTAALGCLVKDYFPEPVTVSWNSGALTSGVHTFPAVLQSSGLYSLSSVVTVPSSSLGTQTYICNVNHKPSNTKVDKKVEPKSCDKTHTCPPCPAPEAAGGPSVFLFPPKPKDTLMISRTPEVTCVVVDVSHEDPEVKFNWYVDGVEVHNAKTKPREEQYNSTYRVVSVLTVLHQDWLNGKEYKCKVSNKALPAPIEKTISKAKGQPREPQVYTLPPCREEMTKNQVSLWCLVKGFYPSDIAVEWESNGQPENNYKTTPPVLDSDGSFFLYSKLTVDKSRWQQGNVFSCSVMHEALHNHYTQKSLSLSPGK

SEQ ID NO: 26 - protein, 708 aa, synthetic construct
QVQLVQSGAEVKKPGASVKVSCKASGYSFTGYYMHWVRQAPGQGLEWIGRINPYNGATTYSQNFKDRATMTVDTSISTAYMELSRLRSDDTAVYYCVPTGMGYFLMDYWGQGTLVTVSSASTKGPSVFPLAPSSKSTSGGTAALGCLVKDYFPEPVTVSWNSGALTSGVHTFPAVLQSSGLYSLSSVVTVPSSSLGTQTYICNVNHKPSNTKVDKKVEPKSCDKTHTCPPCPAPEAAGGPSVFLFPPKPKDTLMISRTPEVTCVVVDVSHEDPEVKFNWYVDGVEVHNAKTKPREEQYNSTYRVVSVLTVLHQDWLNGKEYKCKVSNKALPAPIEKTISKAKGQPREPQVYTLPPCREEMTKNQVSLWCLVKGFYPSDIAVEWESNGQPENNYKTTPPVLDSDGSFFLYSKLTVDKSRWQQGNVFSCSVMHEALHNHYTQKSLSLSPGKGGGGSGGGGSEVQLLESGGGLVQPGGSLKLSCAASGFTFNTYAMNWVRQAPGKGLEWVARIRSKYNNYATYYADSVKDRFTISRDDSKNTAYLQMNNLKTEDTAVYYCVRHGNFGNSYVSWFAYWGQGTLVTVSSGGGGSGGGGSGGGGSELVVTQEPSLTVSPGGTVTLTCRSSTGAVTTSNYANWVQQKPGQAPRGLIGGTNKRAPGTPARFSGSLLGGKAALTLSGVQPEDEAEYYCALWYSNLWVFGGGTKLTVL

SEQ ID NO: 27 - protein, 708 aa, synthetic construct
QVQLVQSGAEVKKPGASVKVSCKASGYSFTGYYMHWVRQAPGQGLEWIGRINPYNGATTYSQNFKDRATMTVDTSISTAYMELSRLRSDDTAVYYCVPTGMGYFLMDYWGQGTLVTVSSASTKGPSVFPLAPSSKSTSGGTAALGCLVKDYFPEPVTVSWNSGALTSGVHTFPAVLQSSGLYSLSSVVTVPSSSLGTQTYICNVNHKPSNTKVDKKVEPKSCDKTHTCPPCPAPEAAGGPSVFLFPPKPKDTLMISRTPEVTCVVVDVSHEDPEVKFNWYVDGVEVHNAKTKPREEQYNSTYRVVSVLTVLHQDWLNGKEYKCKVSNKALPAPIEKTISKAKGQPREPQVCTLPPSREEMTKNQVSLSCAVKGFYPSDIAVEWESNGQPENNYKTTPPVLDSDGSFFLVSKLTVDKSRWQQGNVFSCSVMHEALHNHYTQKSLSLSPGKGGGGSGGGGSEVQLLESGGGLVQPGGSLKLSCAASGFTFNTYAMNWVRQAPGKGLEWVARIRSKYNNYATYYADSVKDRFTISRDDSKNTAYLQMNNLKTEDTAVYYCVRHGNFGNSYVSWFAYWGQGTLVTVSSGGGGSGGGGSGGGGSELVVTQEPSLTVSPGGTVTLTCRSSTGAVTTSNYANWVQQKPGQAPRGLIGGTNKRAPGTPARFSGSLLGGKAALTLSGVQPEDEAEYYCALWYSNLWVFGGGTKLTVL

SEQ ID NO: 28 - protein, 453 aa, synthetic construct
QVQLVQSGAEVKKPGSSVKVSCKTSGDTFSTYAISWVRQAPGQGLEWMGGIIPIFGKAHYAQKFQGRVTITADESTSTAYMELSSLRSEDTAVYFCARKFHFVSGSPFGMDVWGQGTTVTVSSASTKGPSVFPLAPSSKSTSGGTAALGCLVKDYFPEPVTVSWNSGALTSGVHTFPAVLQSSGLYSLSSVVTVPSSSLGTQTYICNVNHKPSNTKVDKKVEPKSCDKTHTCPPCPAPEAAGGPSVFLFPPKPKDTLMISRTPEVTCVVVDVSHEDPEVKFNWYVDGVEVHNAKTKPREEQYNSTYRVVSVLTVLHQDWLNGKEYKCKVSNKALPAPIEKTISKAKGQPREPQVYTLPPSREEMTKNQVSLTCLVKGFYPSDIAVEWESNGQPENNYKTTPPVLDSDGSFFLYSKLTVDKSRWQQGNVFSCSVMHEALHNHYTQKSLSLSPGK

SEQ ID NO: 29 - protein, 453 aa, synthetic construct
QVQLVQSGAEVKKPGSSVKVSCKTSGDTFSTYAISWVRQAPGQGLEWMGGIIPIFGKAHYAQKFQGRVTITADESTSTAYMELSSLRSEDTAVYFCARKFHFVSGSPFGMDVWGQGTTVTVSSASTKGPSVFPLAPSSKSTSGGTAALGCLVKDYFPEPVTVSWNSGALTSGVHTFPAVLQSSGLYSLSSVVTVPSSSLGTQTYICNVNHKPSNTKVDKKVEPKSCDKTHTCPPCPAPEAAGGPSVFLFPPKPKDTLMISRTPEVTCVVVDVSHEDPEVKFNWYVDGVEVHNAKTKPREEQYNSTYRVVSVLTVLHQDWLNGKEYKCKVSNKALPAPIEKTISKAKGQPREPQVCTLPPSREEMTKNQVSLSCAVKGFYPSDIAVEWESNGQPENNYKTTPPVLDSDGSFFLVSKLTVDKSRWQQGNVFSCSVMHEALHNHYTQKSLSLSPGK

SEQ ID NO: 30 - protein, 213 aa, synthetic construct
EIVLTQSPATLSLSPGERATLSCRASQSVSSYLAWYQQKPGQAPRLLIYDASNRATGIPARFSGSGSGTDFTLTISSLEPEDFAVYYCQQRSNWPTFGQGTKVEIKRTVAAPSVFIFPPSDEQLKSGTASVVCLLNNFYPREAKVQWKVDNALQSGNSQESVTEQDSKDSTYSLSSTLTLSKADYEKHKVYACEVTHQGLSSPVTKSFNRGEC

SEQ ID NO: 31 - protein, 449 aa, synthetic construct
EVQLQQSGPDLVKPGASVKISCKASGYSFTGYYMHWVKQSHVKSLEWIGRINPYNGATTYSQNFKDKASLTVDKSSSTAYMELHSLTSEDSAVYYCVPTGMGYFLMDYWGQGTSVTVSSASTKGPSVFPLAPSSKSTSGGTAALGCLVKDYFPEPVTVSWNSGALTSGVHTFPAVLQSSGLYSLSSVVTVPSSSLGTQTYICNVNHKPSNTKVDKKVEPKSCDKTHTCPPCPAPEAAGGPSVFLFPPKPKDTLMISRTPEVTCVVVDVSHEDPEVKFNWYVDGVEVHNAKTKPREEQYNSTYRVVSVLTVLHQDWLNGKEYKCKVSNKALPAPIEKTISKAKGQPREPQVYTLPPSREEMTKNQVSLTCLVKGFYPSDIAVEWESNGQPENNYKTTPPVLDSDGSFFLYSKLTVDKSRWQQGNVFSCSVMHEALHNHYTQKSLSLSPGK

SEQ ID NO: 32 - protein, 213 aa, synthetic construct
DIVMTQSHKFMSASVGDRVSITCKASQDVGSAVVWYRQKPGQSPKLLIYWASTRHTGVPDRFTGSGSGTDFTLTISNVQSEDLADYFCQQFTSYPTFGSGTRLEIKRTVAAPSVFIFPPSDEQLKSGTASVVCLLNNFYPREAKVQWKVDNALQSGNSQESVTEQDSKDSTYSLSSTLTLSKADYEKHKVYACEVTHQGLSSPVTKSFNRGEC